European Patent Specification EP 3 723 479 B1, published May 22, 2024. Title: Methods and compounds for use in the methods. Applicant: ACD Pharmaceuticals AS. The sequence listing filed with the application follows.

SEQUENCE LISTING (6 sequences)

SEQ ID NO: 1 - DNA, 16 bp, Salmo salar
ttgaacgctcctccat

SEQ ID NO: 2 - DNA, 16 bp, Salmo salar
ggagcagcgaggaggt

SEQ ID NO: 3 - DNA, 16 bp, Salmo salar
gcaaaacatttaagta

SEQ ID NO: 4 - DNA, 16 bp, Salmo salar
gctcccttcaatccaa

SEQ ID NO: 5 - DNA, 21 bp, Salmo salar
gagcgttcaagtcaggtgttg

SEQ ID NO: 6 - DNA, 20 bp, Salmo salar
cagagctgacgtttctccgt